European Patent Application EP 4 755 920 A1, published June 10, 2026. Title: 抗IL4R抗体及其应用. Applicant: 先声药业有限公司. Application CN. The sequence listing filed with the application follows.

SEQUENCE LISTING (166 sequences)

SEQ ID NO: 1 - protein, 439 aa, synthetic construct
MKVLQEPTCVSDYMSISTCEWKMNGPTNCSTELRLLYQLVFLLSEAHTCIPENNGGAGCVCHLLMDDVVSADNYTLDLWAGQQLLWKGSFKPSEHVKPRAPGNLTVHTNVSDTLLLTWSNPYPPDNYLYNHLTYAVNIWSENDPADFRIYNVTYLEPSLRIAASTLKSGISYRARVRAWAQCYNTTWSEWSPSTKWHNSYREPFEQHEPKSSDKTHTCPPCPAPELLGGPSVFLFPPKPKDTLMISRTPEVTCVVVDVSHEDPEVKFNWYVDGVEVHNAKTKPREEQYNSTYRVVSVLTVLHQDWLNGKEYKCKVSNKALPAPIEKTISKAKGQPREPQVYTLPPSREEMTKNQVSLTCLVKGFYPSDIAVEWESNGQPENNYKTTPPVLDSDGSFFLYSKLTVDKSRWQQGNVFSCSVMHEALHNHYTQKSLSLSPGK

SEQ ID NO: 2 - protein, 440 aa, synthetic construct
MKVLQEPTCVSDYMSISTCEWKMNGPTNCSTELRLLYQLVFLLSEAHTCIPENNGGAGCVCHLLMDDVVSADNYTLDLWAGQQLLWKGSFKPSEHVKPRAPGNLTVHTNVSDTLLLTWSNPYPPDNYLYNHLTYAVNIWSENDPADFRIYNVTYLEPSLRIAASTLKSGISYRARVRAWAQCYNTTWSEWSPSTKWHNSYREPFEQHEPRGPTIKPCPPCKCPAPNLLGGPSVFIFPPKIKDVLMISLSPIVTCVVVDVSEDDPDVQISWFVNNVEVHTAQTQTHREDYNSTLRVVSALPIQHQDWMSGKEFKCKVNNKDLPAPIERTISKPKGSVRAPQVYVLPPPEEEMTKKQVTLTCMVTDFMPEDIYVEWTNNGKTELNYKNTEPVLDSDGSYFMYSKLRVEKKNWVERNSYSCSVVHEGLHNHHTTKSFSRTPGK

SEQ ID NO: 3 - protein, 213 aa, synthetic construct
MKVLQEPTCVSDYMSISTCEWKMNGPTNCSTELRLLYQLVFLLSEAHTCIPENNGGAGCVCHLLMDDVVSADNYTLDLWAGQQLLWKGSFKPSEHVKPRAPGNLTVHTNVSDTLLLTWSNPYPPDNYLYNHLTYAVNIWSENDPADFRIYNVTYLEPSLRIAASTLKSGISYRARVRAWAQCYNTTWSEWSPSTKWHNSYREPFEQHHHHHHH

SEQ ID NO: 4 - protein, 215 aa, synthetic construct
GSMKVLQEPACVSDYMSISTCEWKMGGPTNCSAELRLLYQLVFQSSETHTCVPENNGGVGCVCHLLMDDVVSMDNYTLDLWAGQQLLWKGSFKPSEHVKPRAPGNLTVHTNVSDTVLLTWSNPYPPDNYLYNDLTYAVNIWSENDPAYSRIHNVTYLKPTLRIPASTLKSGISYRARVRAWAQHYNTTWSEWSPSTKWYNSYREPFEQRHHHHHH

SEQ ID NO: 5 - protein, 825 aa, synthetic construct
MGWLCSGLLFPVSCLVLLQVASSGNMKVLQEPTCVSDYMSISTCEWKMNGPTNCSTELRLLYQLVFLLSEAHTCIPENNGGAGCVCHLLMDDVVSADNYTLDLWAGQQLLWKGSFKPSEHVKPRAPGNLTVHTNVSDTLLLTWSNPYPPDNYLYNHLTYAVNIWSENDPADFRIYNVTYLEPSLRIAASTLKSGISYRARVRAWAQCYNTTWSEWSPSTKWHNSYREPFEQHLLLGVSVSCIVILAVCLLCYVSITKIKKEWWDQIPNPARSRLVAIIIQDAQGSQWEKRSRGQEPAKCPHWKNCLTKLLPCFLEHNMKRDEDPHKAAKEMPFQGSGKSAWCPVEISKTVLWPESISVVRCVELFEAPVECEEEEEVEEEKGSFCASPESSRDDFQEGREGIVARLTESLFLDLLGEENGGFCQQDMGESCLLPPSGSTSAHMPWDEFPSAGPKEAPPWGKEQPLHLEPSPPASPTQSPDNLTCTETPLVIAGNPAYRSFSNSLSQSPCPRELGPDPLLARHLEEVEPEMPCVPQLSEPTTVPQPEPETWEQILRRNVLQHGAAAAPVSAPTSGYQEFVHAVEQGGTQASAVVGLGPPGEAGYKAFSSLLASSAVSPEKCGFGASSGEEGYKPFQDLIPGCPGDPAPVPVPLFTFGLDREPPRSPQSSHLPSSSPEHLGLEPGEKVEDMPKPPLPQEQATDPLVDSLGSGIVYSALTCHLCGHLKQCHGQEDGGQTPVMASPCCGCCCGDRSSPPTTPLRAPDPSPGGVPLEASLCPASLAPSGISEKSKSSSSFHPAPGNAQSSSQTPKIVNFVSVGPTYMRVS

SEQ ID NO: 6 - protein, 125 aa, synthetic construct [sequence omitted]

SEQ ID NO: 7 - protein, 112 aa, synthetic construct [sequence omitted]

SEQ ID NO: 8 - protein, 825 aa, synthetic construct
MGWLCSGLLFPVSCLVLLQVASSGSMKVLQEPACVSDYMSISTCEWKMGGPTNCSAELRLLYQLVFQSSETHTCVPENNGGVGCVCHLLMDDVVSMDNYTLDLWAGQQLLWKGSFKPSEHVKPRAPGNLTVHTNVSDTVLLTWSNPYPPDNYLYNDLTYAVNIWSENDPAYSRIHNVTYLKPTLRIPASTLKSGISYRARVRAWAQHYNTTWSEWSPSTKWYNSYREPFEQRLLWGVSAACVFILFFCLSCYFSVTKIKKEWWDQIPNPARSHLVAIIIQDAQESQWEKRSRGQEAAKCPYWKNCLTKLLPCFLEHNMKRDEDPHKAVKDLPFRGSGKSAWCPVEISKTVLWPESISVVRCVELFEAPVECKEEEEVEEEKGSFCTSSESNRDDFQEGREGIVARLTESLFLDLLGGENGGFFQQDMGESCLLPPLGSTSAHVPWDEFPSAGPKEVPPWGKEQPLHQEPSPPASPTQSPDNPTCTEMPLVISSNPAYRSFSNSLSQSPCPRELGPDPLLARHLEEVDPEMPCAPQLSEPTTVAPAEPETWEQILRRNVLQHGAAAAPASAPTSGYREFVHAVQQGGIQASAVAGLGPPGEAGYKAFSSLLASSAVSPGECGFGASSGEEGYKPFQDLTPGCPGDPAPVPVPLFTFGLDREPPHSPQSSHLPSNSPEHLALEPGEKVEDMQKPPLPPEQATDPLGDNLGSGIVYSALTCHLCGHLKQCHGQEDGGQAPVVASPCCGCCCGDRSSPPTTPLRAPDPSLGGVPLEASLCLASLAPSGISEKSKSSLSFHPAPGSAQSSSQTPQIVNFVSVGPTCMRVS

SEQ ID NO: 9 - protein, 170 aa, synthetic construct
VFTLEDFVGDWRQTAGYNLDQVLEQGGVSSLFQNLGVSVTPIQRIVLSGENGLKIDIHVIIPYEGLSGDQMGQIEKIFKVVYPVDDHHFKVILHYGTLVIDGVTPNMIDYFGRPYEGIAVFDGKKITVTGTLWNGNKIIDERLINPDGSLLFRVTINGVTGWRLCERILA

SEQ ID NO: 10 - protein, 120 aa, synthetic construct
DVQLQESGPGLVKPSQSLSLTCTVTGYSITSDYAWNWIRQFPGNKLEWMGYISYSGSSSYNPSLKSRISITRDTSKNQFFLQLNSVTTDDTATYYCAGGGLRRRGLFDYWGQGTTLTVSS

SEQ ID NO: 11 - protein, 121 aa, synthetic construct
QVQLQQSGAELVKPGASVKLSCKASGYTFTEYTIHWVKQRSGQGLEWIGWFYPGRGSIKYNEKFKDKATLTADKSSSTVYMELSRLTSEDSAVYFCTRHEYRGSNYAMDYWGQGTSVTVSS

SEQ ID NO: 12 - protein, 120 aa, synthetic construct
EVQLQQSGPVLVKPGASVKMSCKASGYTFTDYYMNWVKQRHGKSLDWIGTINPYNGGTGYNQKFKGKATLTVDKSSSTAYMELNSLTSEDSAVYFCARSLLRRRGAMDYWGQGTSVTVSS

SEQ ID NO: 13 - protein, 117 aa, synthetic construct
EVMLVESGGGLVKPGGSLKLSCAASGFTFSSYAMSWVRQTPEKRLEWVAIISGGGDSTYYPDSVKGRFTISRDNAKNTLYLQMSSLRSEDTALYFCARLHYWYFDFWGTGTTVTVSS

SEQ ID NO: 14 - protein, 121 aa, synthetic construct
QAYLQQSGAELVRPGASVKMSCKASGYTFTSYNMHWAKQTPRQGLEWIGSIYPGNGDTSYNQKFKGKATLTVDKSSSTAYMQLSSLTSEDSAVYFCARGGRLRRGDWFAYWGQGTLVTVSA

SEQ ID NO: 15 - protein, 118 aa, synthetic construct
QVQLKQSGPGLVQPSQSLSVTCTVSGFSLTNYGVHWVRQSPGKGLEWLGVIWSGGSTDYNAAFKSRLSISKDNSKSQVFFKMNSLQADDTAIYYCARNKGTRPVFDYWGQGTTLTVSS

SEQ ID NO: 16 - protein, 106 aa, synthetic construct
QIVLSQSPAILSASPGEKVTMTCRATSSVTYMHWYQQKPGSSPKPWIYATSNLASGVPARFSGSGSGTSYSLTISRVEAEDTATYYCQQWSSIPLTFGAGTKLELK

SEQ ID NO: 17 - protein, 112 aa, synthetic construct
DVLMTQTPLSLPVSLGDQASISCRSSQSIVHSSGNTYLQWYLQKPGQSPKLLIYKVSNRFSGVPDRFSGSGSGTDFTLKISRVEAEDLGVYYCFQGSHVPPTFGGGTKLEIK

SEQ ID NO: 18 - protein, 110 aa, synthetic construct
DIVLTQSPASLVVSLGQRATISCRASKSVSTSGYGYIHWYRQKPGQPPKLLIYLVSNLESGVPARFSGSGSGTDFTLNIHPVEEEDAATYYCQHIRELYTFGGGTKLEIK

SEQ ID NO: 19 - protein, 107 aa, synthetic construct
DIQMTQSSSSFSVSLGDRVTITCKASEDLYNRLAWYQQKPGNAPRLLISGATSLETGVPSRFSGSGSGRDYTLIITSLQTEDVATYYCQQYWRNPYTFGGGTKLEIK

SEQ ID NO: 20 - protein, 107 aa, synthetic construct
DIQMTQSPASLSASVGETVTITCRASENIYSYLIWYQQKQGKSPQLLVYDAKTLAEGVPSRFSGSGSGSQFSLKINSLQPEDFGTYYCQHHYGTPLTFGGGTKLELK

SEQ ID NO: 21 - protein, 106 aa, synthetic construct
DIQMTQSPASLSASVGETVTITCRASENIYSYLAWYQQKQGKSPQLLVYNAKTLAEGVPSRFSGSGSGTQFSLKINSLQPEDFGSYYCQHYVSPLTFGAGTKLEVK

SEQ ID NO: 22 - protein, 6 aa, synthetic construct
SDYAWN

SEQ ID NO: 23 - protein, 16 aa, synthetic construct
YISYSGSSSYNPSLKS

SEQ ID NO: 24 - protein, 11 aa, synthetic construct
GGLRRRGLFDY

SEQ ID NO: 25 - protein, 9 aa, synthetic construct
GYSITSDYA

SEQ ID NO: 26 - protein, 7 aa, synthetic construct
ISYSGSS

SEQ ID NO: 27 - protein, 13 aa, synthetic construct
AGGGLRRRGLFDY

SEQ ID NO: 28 - protein, 8 aa, synthetic construct
GYSITSDY

SEQ ID NO: 29 - protein, 5 aa, synthetic construct
SYSGS

SEQ ID NO: 30 - protein, 11 aa, synthetic construct
GGLRRRGLFDY

SEQ ID NO: 31 - protein, 5 aa, synthetic construct
EYTIH

SEQ ID NO: 32 - protein, 17 aa, synthetic construct
WFYPGRGSIKYNEKFKD

SEQ ID NO: 33 - protein, 12 aa, synthetic construct
HEYRGSNYAMDY

SEQ ID NO: 34 - protein, 8 aa, synthetic construct
GYTFTEYT

SEQ ID NO: 35 - protein, 8 aa, synthetic construct
FYPGRGSI

SEQ ID NO: 36 - protein, 14 aa, synthetic construct
TRHEYRGSNYAMDY

SEQ ID NO: 37 - protein, 7 aa, synthetic construct
GYTFTEY

SEQ ID NO: 38 - protein, 6 aa, synthetic construct
YPGRGS

SEQ ID NO: 39 - protein, 12 aa, synthetic construct
HEYRGSNYAMDY

SEQ ID NO: 40 - protein, 5 aa, synthetic construct
DYYMN

SEQ ID NO: 41 - protein, 17 aa, synthetic construct
TINPYNGGTGYNQKFKG

SEQ ID NO: 42 - protein, 11 aa, synthetic construct
SLLRRRGAMDY

SEQ ID NO: 43 - protein, 8 aa, synthetic construct
GYTFTDYY

SEQ ID NO: 44 - protein, 8 aa, synthetic construct
INPYNGGT

SEQ ID NO: 45 - protein, 13 aa, synthetic construct
ARSLLRRRGAMDY

SEQ ID NO: 46 - protein, 7 aa, synthetic construct
GYTFTDY

SEQ ID NO: 47 - protein, 6 aa, synthetic construct
NPYNGG

SEQ ID NO: 48 - protein, 11 aa, synthetic construct
SLLRRRGAMDY

SEQ ID NO: 49 - protein, 5 aa, synthetic construct
SYAMS

SEQ ID NO: 50 - protein, 17 aa, synthetic construct
IISGGGDSTYYPDSVKG

SEQ ID NO: 51 - protein, 8 aa, synthetic construct
LHYWYFDF

SEQ ID NO: 52 - protein, 8 aa, synthetic construct
GFTFSSYA

SEQ ID NO: 53 - protein, 8 aa, synthetic construct
ISGGGDST

SEQ ID NO: 54 - protein, 10 aa, synthetic construct
ARLHYWYFDF

SEQ ID NO: 55 - protein, 7 aa, synthetic construct
GFTFSSY

SEQ ID NO: 56 - protein, 6 aa, synthetic construct
SGGGDS

SEQ ID NO: 57 - protein, 8 aa, synthetic construct
LHYWYFDF

SEQ ID NO: 58 - protein, 5 aa, synthetic construct
SYNMH

SEQ ID NO: 59 - protein, 17 aa, synthetic construct
SIYPGNGDTSYNQKFKG

SEQ ID NO: 60 - protein, 12 aa, synthetic construct
GGRLRRGDWFAY

SEQ ID NO: 61 - protein, 8 aa, synthetic construct
GYTFTSYN

SEQ ID NO: 62 - protein, 8 aa, synthetic construct
IYPGNGDT

SEQ ID NO: 63 - protein, 14 aa, synthetic construct
ARGGRLRRGDWFAY

SEQ ID NO: 64 - protein, 7 aa, synthetic construct
GYTFTSY

SEQ ID NO: 65 - protein, 6 aa, synthetic construct
YPGNGD

SEQ ID NO: 66 - protein, 12 aa, synthetic construct
GGRLRRGDWFAY

SEQ ID NO: 67 - protein, 5 aa, synthetic construct
NYGVH

SEQ ID NO: 68 - protein, 16 aa, synthetic construct
VIWSGGSTDYNAAFKS

SEQ ID NO: 69 - protein, 10 aa, synthetic construct
NKGTRPVFDY

SEQ ID NO: 70 - protein, 8 aa, synthetic construct
GFSLTNYG

SEQ ID NO: 71 - protein, 7 aa, synthetic construct
IWSGGST

SEQ ID NO: 72 - protein, 12 aa, synthetic construct
ARNKGTRPVFDY

SEQ ID NO: 73 - protein, 7 aa, synthetic construct
GFSLTNY

SEQ ID NO: 74 - protein, 5 aa, synthetic construct
WSGGS

SEQ ID NO: 75 - protein, 10 aa, synthetic construct
NKGTRPVFDY

SEQ ID NO: 76 - protein, 10 aa, synthetic construct
RATSSVTYMH

SEQ ID NO: 77 - protein, 7 aa, synthetic construct
ATSNLAS

SEQ ID NO: 78 - protein, 9 aa, synthetic construct
QQWSSIPLT

SEQ ID NO: 79 - protein, 5 aa, synthetic construct
SSVTY

SEQ ID NO: 80 - skipped

SEQ ID NO: 81 - protein, 9 aa, synthetic construct
QQWSSIPLT

SEQ ID NO: 82 - protein, 10 aa, synthetic construct
RATSSVTYMH

SEQ ID NO: 83 - protein, 7 aa, synthetic construct
ATSNLAS

SEQ ID NO: 84 - protein, 9 aa, synthetic construct
QQWSSIPLT

SEQ ID NO: 85 - protein, 16 aa, synthetic construct
RSSQSIVHSSGNTYLQ

SEQ ID NO: 86 - protein, 7 aa, synthetic construct
KVSNRFS

SEQ ID NO: 87 - protein, 9 aa, synthetic construct
FQGSHVPPT

SEQ ID NO: 88 - protein, 11 aa, synthetic construct
QSIVHSSGNTY

SEQ ID NO: 89 - skipped

SEQ ID NO: 90 - protein, 9 aa, synthetic construct
FQGSHVPPT

SEQ ID NO: 91 - protein, 16 aa, synthetic construct
RSSQSIVHSSGNTYLQ

SEQ ID NO: 92 - protein, 7 aa, synthetic construct
KVSNRFS

SEQ ID NO: 93 - protein, 9 aa, synthetic construct
FQGSHVPPT

SEQ ID NO: 94 - protein, 15 aa, synthetic construct
RASKSVSTSGYGYIH

SEQ ID NO: 95 - protein, 7 aa, synthetic construct
LVSNLES

SEQ ID NO: 96 - protein, 8 aa, synthetic construct
QHIRELYT

SEQ ID NO: 97 - protein, 10 aa, synthetic construct
KSVSTSGYGY

SEQ ID NO: 98 - skipped

SEQ ID NO: 99 - protein, 8 aa, synthetic construct
QHIRELYT

SEQ ID NO: 100 - protein, 15 aa, synthetic construct
RASKSVSTSGYGYIH

SEQ ID NO: 101 - protein, 7 aa, synthetic construct
LVSNLES

SEQ ID NO: 102 - protein, 8 aa, synthetic construct
QHIRELYT

SEQ ID NO: 103 - protein, 11 aa, synthetic construct
KASEDLYNRLA

SEQ ID NO: 104 - protein, 7 aa, synthetic construct
GATSLET

SEQ ID NO: 105 - protein, 9 aa, synthetic construct
QQYWRNPYT

SEQ ID NO: 106 - protein, 6 aa, synthetic construct
EDLYNR

SEQ ID NO: 107 - skipped

SEQ ID NO: 108 - protein, 9 aa, synthetic construct
QQYWRNPYT

SEQ ID NO: 109 - protein, 11 aa, synthetic construct
KASEDLYNRLA

SEQ ID NO: 110 - protein, 7 aa, synthetic construct
GATSLET

SEQ ID NO: 111 - protein, 9 aa, synthetic construct
QQYWRNPYT

SEQ ID NO: 112 - protein, 11 aa, synthetic construct
RASENIYSYLI

SEQ ID NO: 113 - protein, 7 aa, synthetic construct
DAKTLAE

SEQ ID NO: 114 - protein, 9 aa, synthetic construct
QHHYGTPLT

SEQ ID NO: 115 - protein, 6 aa, synthetic construct
ENIYSY

SEQ ID NO: 116 - skipped

SEQ ID NO: 117 - protein, 9 aa, synthetic construct
QHHYGTPLT

SEQ ID NO: 118 - protein, 11 aa, synthetic construct
RASENIYSYLI

SEQ ID NO: 119 - protein, 7 aa, synthetic construct
DAKTLAE

SEQ ID NO: 120 - protein, 9 aa, synthetic construct
QHHYGTPLT

SEQ ID NO: 121 - protein, 11 aa, synthetic construct
RASENIYSYLA

SEQ ID NO: 122 - protein, 7 aa, synthetic construct
NAKTLAE

SEQ ID NO: 123 - protein, 8 aa, synthetic construct
QHYVSPLT

SEQ ID NO: 124 - protein, 6 aa, synthetic construct
ENIYSY

SEQ ID NO: 125 - skipped

SEQ ID NO: 126 - protein, 8 aa, synthetic construct
QHYVSPLT

SEQ ID NO: 127 - protein, 11 aa, synthetic construct
RASENIYSYLA

SEQ ID NO: 128 - protein, 7 aa, synthetic construct
NAKTLAE

SEQ ID NO: 129 - protein, 8 aa, synthetic construct
QHYVSPLT

SEQ ID NO: 130 - protein, 95 aa, synthetic construct
DIQLTQSPSFLSASVGDRVTITCRASQGISSYLAWYQQKPGKAPKLLIYAASTLQSGVPSRFSGSGSGTEFTLTISSLQPEDFATYYCQQLNSYP

SEQ ID NO: 131 - protein, 10 aa, synthetic construct
FGQGTKLEIK

SEQ ID NO: 132 - protein, 98 aa, synthetic construct
QVQLQESGPGLVKPSETLSLTCTVSGYSISSGYYWGWIRQPPGKGLEWIGSIYHSGSTYYNPSLKSRVTISVDTSKNQFSLKLSSVTAADTAVYYCAR

SEQ ID NO: 133 - protein, 11 aa, synthetic construct
WGQGTTVTVSS

SEQ ID NO: 134 - protein, 106 aa, synthetic construct
DIQLTQSPSFLSASVGDRVTITCRATSSVTYMHWYQQKPGKAPKPWIYATSNLASGVPSRFSGSGSGTEFTLTISSLQPEDFATYYCQQWSSIPLTFGQGTKLEIK

SEQ ID NO: 135 - protein, 120 aa, synthetic construct
EVQLQESGPGLVKPSETLSLTCTVSGYSISSDYAWNWIRQPPGKGLEWIGYISYSGSSSYNPSLKSRVTISRDTSKNQFSLKLSSVTAADTAVYYCAGGGLRRRGLFDYWGQGTTVTVSS

SEQ ID NO: 136 - protein, 120 aa, synthetic construct
EVQLQESGPGLVKPSETLSLTCTVSGYSISSDYAWNWIRQPPGKGLEWIGYISYSGSSSYNPSLKSRVTISVDTSKNQFSLKLSSVTAADTAVYYCARGGLRRRGLFDYWGQGTTVTVSS

SEQ ID NO: 137 - protein, 101 aa, synthetic construct
DIVMTQSPDSLAVSLGERATINCKSSQSVLYSSNNKNYLAWYQQKPGQPPKLLIYWASTRESGVPDRFSGSGSGTDFTLTISSLQAEDVAVYYCQQYYSTP

SEQ ID NO: 138 - protein, 10 aa, synthetic construct
FGGGTKVEIK

SEQ ID NO: 139 - protein, 98 aa, synthetic construct
QVQLVQSGAEVKKPGSSVKVSCKASGGTFSSYTISWVRQAPGQGLEWMGRIIPILGIANYAQKFQGRVTITADKSTSTAYMELSSLRSEDTAVYYCAR

SEQ ID NO: 140 - protein, 112 aa, synthetic construct
DIVMTQSPDSLAVSLGERATINCRSSQSIVHSSGNTYLQWYQQKPGQSPKLLIYKVSNRFSGVPDRFSGSGSGTDFTLTISSLQAEDVAVYYCFQGSHVPPTFGGGTKVEIK

SEQ ID NO: 141 - protein, 121 aa, synthetic construct
EVQLVQSGAEVKKPGSSVKVSCKASGYTFSEYTIHWVRQAPGQGLEWMGWFYPGRGSIKYNEKFKDRVTITADKSTSTAYMELSSLRSEDTAVYYCTRHEYRGSNYAMDYWGQGTTVTVSS

SEQ ID NO: 142 - protein, 121 aa, synthetic construct
EVQLVQSGAEVKKPGSSVKVSCKASGYTFTEYTIHWVRQAPGQGLEWMGWFYPGRGSIKYNEKFKDRVTITADKSTSTAYMELSSLRSEDTAVYYCTRHEYRGSNYAMDYWGQGTTVTVSS

SEQ ID NO: 143 - protein, 121 aa, synthetic construct
EVQLVQSGAEVKKPGSSVKVSCKASGYTFTEYTIHWVRQAPGQGLEWMGWFYPGRGSIKYNEKFKDRVTITADKSTSTVYMELSSLRSEDTAVYYCTRHEYRGSNYAMDYWGQGTTVTVSS

SEQ ID NO: 144 - protein, 98 aa, synthetic construct
QVQLVQSGAEVKKPGASVKVSCKASGYTFTSYAMHWVRQAPGQRLEWMGWINAGNGNTKYSQKFQGRVTITRDTSASTAYMELSSLRSEDTAVYYCAR

SEQ ID NO: 145 - protein, 110 aa, synthetic construct
DIVLTQSPDSLAVSLGERATINCRASKSVSTSGYGYIHWYQQKPGQPPKLLIYLVSNLESGVPDRFSGSGSGTDFTLTISSLQAEDVATYYCQHIRELYTFGGGTKVEIK

SEQ ID NO: 146 - protein, 110 aa, synthetic construct
DIVLTQSPDSLAVSLGERATINCRASKSVSTSGYGYIHWYQQKPGQPPKLLIYLVDNLESGVPDRFSGSGSGTDFTLTISSLQAEDVATYYCQHIRELYTFGGGTKVEIK

SEQ ID NO: 147 - protein, 120 aa, synthetic construct
EVQLVQSGAEVKKPGASVKVSCKASGYTFTDYYMNWVRQAPGQRLEWMGTINPYNAGTGYNQKFKGRVTITVDKSASTAYMELSSLRSEDTAVYYCARSLLRRRGAMDYWGQGTTVTVSS

SEQ ID NO: 148 - protein, 120 aa, synthetic construct
EVQLVQSGAEVKKPGASVKVSCKASGYTFTDYYMNWVRQAPGKRLEWMGTINPYNAGTGYNQKFKGRVTITVDKSASTAYMELSSLRSEDTAVYYCARSLLRRRGAMDYWGQGTTVTVSS

SEQ ID NO: 149 - protein, 17 aa, synthetic construct
TINPYNAGTGYNQKFKG

SEQ ID NO: 150 - protein, 7 aa, synthetic construct
LVDNLES

SEQ ID NO: 151 - protein, 95 aa, synthetic construct
DIQMTQSPSSLSASVGDRVTITCRASQSISSYLNWYQQKPGKAPKLLIYAASSLQSGVPSRFSGSGSGTDFTLTISSLQPEDFATYYCQQSYSTP

SEQ ID NO: 152 - protein, 98 aa, synthetic construct
EVQLVESGGGLVQPGGSLRLSCAASGFTFSSYWMSWVRQAPGKGLEWVANIKQDGSEKYYVDSVKGRFTISRDNAKNSLYLQMNSLRAEDTAVYYCAR

SEQ ID NO: 153 - protein, 107 aa, synthetic construct
DIQMTQSPSSLSASVGDRVTITCKASEDLYNRLAWYQQKPGKAPKLLISGATSLETGVPSRFSGSGSGRDFTLTISSLQPEDFATYYCQQYWRNPYTFGGGTKVEIK

SEQ ID NO: 154 - protein, 117 aa, synthetic construct
EVQLVESGGGLVQPGGSLRLSCAASGFTFSSYAMSWVRQAPGKGLEWVAIISGGGDSTYYPDSVKGRFTISRDNAKNSLYLQMNSLRAEDTAVYYCARLHYWYFDFWGQGTTVTVSS

SEQ ID NO: 155 - protein, 117 aa, synthetic construct
EVQLVESGGGLVQPGGSLRLSCAASGFTFSSYAMSWVRQAPEKRLEWVAIISGGGDSTYYPDSVKGRFTISRDNAKNSLYLQMNSLRAEDTAVYYCARLHYWYFDFWGQGTTVTVSS

SEQ ID NO: 156 - protein, 100 aa, synthetic construct
DIVMTQSPLSLPVTPGEPASISCRSSQSLLHSNGYNYLDWYLQKPGQSPQLLIYLGSNRASGVPDRFSGSGSGTDFTLKISRVEAEDVGVYYCMQALQTP

SEQ ID NO: 157 - protein, 11 aa, synthetic construct
WGQGTLVTVSS

SEQ ID NO: 158 - protein, 107 aa, synthetic construct
DIQMTQSPSSLSASVGDRVTITCRASENIYSYLIWYQQKPGKSPKLLIYDAKTLAEGVPSRFSGSGSGTDFTLTISSLQPEDFATYYCQHHYGTPLTFGGGTKVEIK

SEQ ID NO: 159 - protein, 107 aa, synthetic construct
DIQMTQSPSSLSASVGDRVTITCRASENIYSYLIWYQQKPGKAPKLLVYDAKTLAEGVPSRFSGSGSGTDFTLTISSLQPEDFATYYCQHHYGTPLTFGGGTKVEIK

SEQ ID NO: 160 - protein, 107 aa, synthetic construct
DIVMTQSPLSLPVTPGEPASISCRASENIYSYLIWYQQKPGQSPQLLIYDAKTLAEGVPDRFSGSGSGTDFTLKISRVEAEDVGVYYCQHHYGTPLTFGGGTKVEIK

SEQ ID NO: 161 - protein, 121 aa, synthetic construct
EVQLVQSGAEVKKPGASVKVSCKASGYTFTSYNMHWARQAPGQRLEWMGSIYPGNGDTSYNQKFKGRVTITVDKSASTAYMELSSLRSEDTAVYYCARGGRLRRGDWFAYWGQGTLVTVSS

SEQ ID NO: 162 - protein, 100 aa, synthetic construct
QVTLKESGPVLVKPTETLTLTCTVSGFSLSNARMGVSWIRQPPGKALEWLAHIFSNDEKSYSTSLKSRLTISKDTSKSQVVLTMTNMDPVDTATYYCARI

SEQ ID NO: 163 - protein, 106 aa, synthetic construct
DIQMTQSPSSLSASVGDRVTITCRASENIYSYLAWYQQKPGKAPKLLIYNAKTLAEGVPSRFSGSGSGTDFTLTISSLQPEDFATYYCQHYVSPLTFGQGTKLEIK

SEQ ID NO: 164 - protein, 118 aa, synthetic construct
EVTLKESGPVLVKPTETLTLTCTVSGFSLTNYGVHWIRQPPGKALEWLGVIWSGGSTDYNAAFKSRLTISKDNSKSQVVLTMTNMDPVDTATYYCARNKGTRPVFDYWGQGTTVTVSS

SEQ ID NO: 165 - protein, 118 aa, synthetic construct
EVTLKESGPVLVKPTETLTLTCTVSGFSLTNYGVHWIRQPPGKALEWLAVIWSGGSTDYNAAFKSRLTISKDNSKSQVFLTMTNMDPVDTATYYCARNKGTRPVFDYWGQGTTVTVSS

SEQ ID NO: 166 - protein, 6 aa, synthetic construct
HHHHHH